European Patent Specification EP 3 498 846 B1, published November 6, 2024. Title: Engineered-immune regulatory factor and Immunity Activation thereby. Applicant: ToolGen Incorporation. The sequence listing filed with the application follows.

SEQUENCE LISTING (289 sequences)

SEQ ID NO: 1 - DNA, 23 bp, Homo Sapiens
cttgtggcgctgaaaacgaacgg

SEQ ID NO: 2 - DNA, 23 bp, Homo Sapiens
atgccacttctcagtacatgtgg

SEQ ID NO: 3 - DNA, 23 bp, Homo Sapiens
gccacttctcagtacatgtgggg

SEQ ID NO: 4 - DNA, 23 bp, Homo Sapiens
gccccacatgtactgagaagtgg

SEQ ID NO: 5 - DNA, 23 bp, Homo Sapiens
tcagtacatgtggggcgttcagg

SEQ ID NO: 6 - DNA, 23 bp, Homo Sapiens
gggcgttcaggacacagacttgg

SEQ ID NO: 7 - DNA, 23 bp, Homo Sapiens
cacagacttggtactgaggaagg

SEQ ID NO: 8 - DNA, 23 bp, Homo Sapiens
ggcgctgttcagcacgctcaagg

SEQ ID NO: 9 - DNA, 23 bp, Homo Sapiens
cacgcaactttaaattccgctgg

SEQ ID NO: 10 - DNA, 23 bp, Homo Sapiens
cggggctttgctatgatactcgg

SEQ ID NO: 11 - DNA, 23 bp, Homo Sapiens
ggcttccacagacacacccatgg

SEQ ID NO: 12 - DNA, 23 bp, Homo Sapiens
tgaagtccacttcgggccatggg

SEQ ID NO: 13 - DNA, 23 bp, Homo sapiens
ctgtacgacacggacagaaatgg

SEQ ID NO: 14 - DNA, 23 bp, Homo Sapiens
tgtacgacacggacagaaatggg

SEQ ID NO: 15 - DNA, 23 bp, Homo Sapiens
cacggacagaaatgggatcctgg

SEQ ID NO: 16 - DNA, 23 bp, Homo Sapiens
gatgcgagtggctgaatacctgg

SEQ ID NO: 17 - DNA, 23 bp, Homo Sapiens
gagtggctgaatacctggattgg

SEQ ID NO: 18 - DNA, 23 bp, Homo Sapiens
agtggctgaatacctggattggg

SEQ ID NO: 19 - DNA, 23 bp, Homo Sapiens
attgggatgtgtctgagctgagg

SEQ ID NO: 20 - DNA, 23 bp, Homo Sapiens
atgaaagagattgactatgatgg

SEQ ID NO: 21 - DNA, 23 bp, Homo Sapiens
ctctgtctctcaagctgagtggg

SEQ ID NO: 22 - DNA, 23 bp, Homo Sapiens
tctctcaagctgagtgggtccgg

SEQ ID NO: 23 - DNA, 23 bp, Homo Sapiens
ctctcaagctgagtgggtccggg

SEQ ID NO: 24 - DNA, 23 bp, Homo Sapiens
caagctgagtgggtccgggctgg

SEQ ID NO: 25 - DNA, 23 bp, Homo Sapiens
ttgacatgactggagagaagagg

SEQ ID NO: 26 - DNA, 23 bp, Homo Sapiens
gactggagagaagaggtcgttgg

SEQ ID NO: 27 - DNA, 23 bp, Homo Sapiens
gagacgggagcaaagctgctggg

SEQ ID NO: 28 - DNA, 23 bp, Homo Sapiens
agagacgggagcaaagctgctgg

SEQ ID NO: 29 - DNA, 23 bp, Homo Sapiens
tggtttctaggtgcagagacggg

SEQ ID NO: 30 - DNA, 23 bp, Homo Sapiens
taagtgaaggtctggtttctagg

SEQ ID NO: 31 - DNA, 23 bp, Homo Sapiens
tgcccatgtaagtgaaggtctgg

SEQ ID NO: 32 - DNA, 23 bp, Homo Sapiens
gaacttgcccatgtaagtgaagg

SEQ ID NO: 33 - DNA, 23 bp, Homo Sapiens
tccattgaccctcagtaccctgg

SEQ ID NO: 34 - DNA, 23 bp, Homo Sapiens
tatgccttctgggtagcagctgg

SEQ ID NO: 35 - DNA, 23 bp, Homo Sapiens
tgagtgcaggcatcttgcaaggg

SEQ ID NO: 36 - DNA, 23 bp, Homo Sapiens
gagtgcaggcatcttgcaagggg

SEQ ID NO: 37 - DNA, 23 bp, Homo Sapiens
gatgaggctgtggttgaagctgg

SEQ ID NO: 38 - DNA, 23 bp, Homo Sapiens
ccactggccacaggacccctggg

SEQ ID NO: 39 - DNA, 23 bp, Homo Sapiens
gggacatggtgcacacacccagg

SEQ ID NO: 40 - DNA, 23 bp, Homo Sapiens
gagtacaggtggtccaggtcagg

SEQ ID NO: 41 - DNA, 23 bp, Homo Sapiens
gcggagagtacaggtggtccagg

SEQ ID NO: 42 - DNA, 23 bp, Homo Sapiens
gcggtggcggagagtacaggtgg

SEQ ID NO: 43 - DNA, 23 bp, Homo Sapiens
tctcctgcacagccagaataagg

SEQ ID NO: 44 - DNA, 23 bp, Homo Sapiens
acgcagaagggtcctggtagagg

SEQ ID NO: 45 - DNA, 23 bp, Homo Sapiens
aggtggtgggtaggccagagagg

SEQ ID NO: 46 - DNA, 23 bp, Homo Sapiens
cccaagccagccacggacccagg

SEQ ID NO: 47 - DNA, 23 bp, Homo Sapiens
acctgggtccgtggctggcttgg

SEQ ID NO: 48 - DNA, 23 bp, Homo Sapiens
aagagacctgggtccgtggctgg

SEQ ID NO: 49 - DNA, 23 bp, Homo Sapiens
ggatcattgggaagagacctggg

SEQ ID NO: 50 - DNA, 23 bp, Homo Sapiens
gggatcattgggaagagacctgg

SEQ ID NO: 51 - DNA, 23 bp, Homo Sapiens
caggatagtctgggatcattggg

SEQ ID NO: 52 - DNA, 23 bp, Homo Sapiens
ggaaagaatccaggatagtctgg

SEQ ID NO: 53 - DNA, 23 bp, Homo Sapiens
cagtgccagagagacctacatgg

SEQ ID NO: 54 - DNA, 23 bp, Homo Sapiens
ctgtaccatgtaggtctctctgg

SEQ ID NO: 55 - DNA, 23 bp, Homo Sapiens
agagacctacatggtacagctgg

SEQ ID NO: 56 - DNA, 23 bp, Homo Sapiens
ctgggccagctgtaccatgtagg

SEQ ID NO: 57 - DNA, 23 bp, Homo Sapiens
agggaaagggcttacggtctggg

SEQ ID NO: 58 - DNA, 23 bp, Homo Sapiens
cagggaaagggcttacggtctgg

SEQ ID NO: 59 - DNA, 23 bp, Homo Sapiens
tctggagatcttcttgcaacagg

SEQ ID NO: 60 - DNA, 23 bp, Homo Sapiens
ctccggttcatgactttgaaagg

SEQ ID NO: 61 - DNA, 23 bp, Homo Sapiens
gtcttccatcttcgtctttcagg

SEQ ID NO: 62 - DNA, 23 bp, Homo Sapiens
gaagacttcgagacccatttagg

SEQ ID NO: 63 - DNA, 23 bp, Homo Sapiens
tcgagacccatttaggatcacgg

SEQ ID NO: 64 - DNA, 23 bp, Homo Sapiens
gtagcgccgtgatcctaaatggg

SEQ ID NO: 65 - DNA, 23 bp, Homo Sapiens
cgtagcgccgtgatcctaaatgg

SEQ ID NO: 66 - DNA, 23 bp, Homo Sapiens
catttaggatcacggcgctacgg

SEQ ID NO: 67 - DNA, 23 bp, Homo Sapiens
ggtcccaatattgaagcccatgg

SEQ ID NO: 68 - DNA, 23 bp, Homo Sapiens
gatccatgggcttcaatattggg

SEQ ID NO: 69 - DNA, 23 bp, Homo Sapiens
agatccatgggcttcaatattgg

SEQ ID NO: 70 - DNA, 23 bp, Homo Sapiens
gcttctaccataagatccatggg

SEQ ID NO: 71 - DNA, 23 bp, Homo Sapiens
cgcttctaccataagatccatgg

SEQ ID NO: 72 - DNA, 23 bp, Homo Sapiens
gcatttgcaaaaattcgccgtgg

SEQ ID NO: 73 - DNA, 23 bp, Homo Sapiens
atgacctgagaattaatttatgg

SEQ ID NO: 74 - DNA, 23 bp, Homo Sapiens
ccatgcactcccagacatcgtgg

SEQ ID NO: 75 - DNA, 23 bp, Homo Sapiens
gcactggtgcgggtggaactcgg

SEQ ID NO: 76 - DNA, 23 bp, Homo Sapiens
acacgttgcactggtgcgggtgg

SEQ ID NO: 77 - DNA, 23 bp, Homo Sapiens
cgaacacgttgcactggtgcggg

SEQ ID NO: 78 - DNA, 23 bp, Homo Sapiens
acgaacacgttgcactggtgcgg

SEQ ID NO: 79 - DNA, 23 bp, Homo Sapiens
tgtagacgaacacgttgcactgg

SEQ ID NO: 80 - DNA, 23 bp, Homo Sapiens
gcgcatgtcacacaggcggatgg

SEQ ID NO: 81 - DNA, 23 bp, Homo Sapiens
aggagcgcatgtcacacaggcgg

SEQ ID NO: 82 - DNA, 23 bp, Homo Sapiens
ccgaggagcgcatgtcacacagg

SEQ ID NO: 83 - DNA, 23 bp, Homo Sapiens
cctgtgtgacatgcgctcctcgg

SEQ ID NO: 84 - DNA, 23 bp, Homo Sapiens
cgactggccagggcgcctgtggg

SEQ ID NO: 85 - DNA, 23 bp, Homo Sapiens
accgcccagacgactggccaggg

SEQ ID NO: 86 - DNA, 23 bp, Homo Sapiens
caccgcccagacgactggccagg

SEQ ID NO: 87 - DNA, 23 bp, Homo Sapiens
gtctgggcggtgctacaactggg

SEQ ID NO: 88 - DNA, 23 bp, Homo Sapiens
ctacaactgggctggcggccagg

SEQ ID NO: 89 - DNA, 23 bp, Homo Sapiens
cacctacctaagaaccatcctgg

SEQ ID NO: 90 - DNA, 23 bp, Homo Sapiens
cggtcaccacgagcagggctggg

SEQ ID NO: 91 - DNA, 23 bp, Homo Sapiens
gccctgctcgtggtgaccgaagg

SEQ ID NO: 92 - DNA, 23 bp, Homo Sapiens
cggagagcttcgtgctaaactgg

SEQ ID NO: 93 - DNA, 23 bp, Homo Sapiens
cagcttgtccgtctggttgctgg

SEQ ID NO: 94 - DNA, 23 bp, Homo Sapiens
aggcggccagcttgtccgtctgg

SEQ ID NO: 95 - DNA, 23 bp, Homo Sapiens
ccgggctggctgcggtcctcggg

SEQ ID NO: 96 - DNA, 23 bp, Homo Sapiens
cgttgggcagttgtgtgacacgg

SEQ ID NO: 97 - DNA, 23 bp, Homo Sapiens
cataaagccatggcttgccttgg

SEQ ID NO: 98 - DNA, 23 bp, Homo Sapiens
ccttggatttcagcggcacaagg

SEQ ID NO: 99 - DNA, 23 bp, Homo Sapiens
ccttgtgccgctgaaatccaagg

SEQ ID NO: 100 - DNA, 23 bp, Homo Sapiens
cactcacctttgcagaagacagg

SEQ ID NO: 101 - DNA, 23 bp, Homo Sapiens
ttccatgctagcaatgcacgtgg

SEQ ID NO: 102 - DNA, 23 bp, Homo Sapiens
ggccacgtgcattgctagcatgg

SEQ ID NO: 103 - DNA, 23 bp, Homo Sapiens
ggcccagcctgctgtggtactgg

SEQ ID NO: 104 - DNA, 23 bp, Homo Sapiens
aggtccgggtgacagtgcttcgg

SEQ ID NO: 105 - DNA, 23 bp, Homo Sapiens
ccgggtgacagtgcttcggcagg

SEQ ID NO: 106 - DNA, 23 bp, Homo Sapiens
ctgtgcggcaacctacatgatgg

SEQ ID NO: 107 - DNA, 23 bp, Homo Sapiens
caactcattccccatcatgtagg

SEQ ID NO: 108 - DNA, 23 bp, Homo Sapiens
ctagatgattccatctgcacggg

SEQ ID NO: 109 - DNA, 23 bp, Homo Sapiens
ggctaggagtcagcgacatatgg

SEQ ID NO: 110 - DNA, 23 bp, Homo Sapiens
gctaggagtcagcgacatatggg

SEQ ID NO: 111 - DNA, 23 bp, Homo Sapiens
ctaggagtcagcgacatatgggg

SEQ ID NO: 112 - DNA, 23 bp, Homo Sapiens
gtactgtgtagccaggatgctgg

SEQ ID NO: 113 - DNA, 23 bp, Homo Sapiens
acgagcactcaccagcatcctgg

SEQ ID NO: 114 - DNA, 23 bp, Homo Sapiens
aggctccaggaatgtccgcgagg

SEQ ID NO: 115 - DNA, 23 bp, Homo Sapiens
acttacctcgcggacattcctgg

SEQ ID NO: 116 - DNA, 23 bp, Homo Sapiens
caccctgggcacttacctcgcgg

SEQ ID NO: 117 - DNA, 23 bp, Homo Sapiens
gtgccgtacaaaggttggctggg

SEQ ID NO: 118 - DNA, 23 bp, Homo Sapiens
ggtgccgtacaaaggttggctgg

SEQ ID NO: 119 - DNA, 23 bp, Homo Sapiens
ctctcctcagtaccacagcaagg

SEQ ID NO: 120 - DNA, 23 bp, Homo Sapiens
cctggggcctccgggcgcggagg

SEQ ID NO: 121 - DNA, 23 bp, Homo Sapiens
agtactcacctggggcctccggg

SEQ ID NO: 122 - DNA, 23 bp, Homo Sapiens
agggtctccagcggccctcctgg

SEQ ID NO: 123 - DNA, 23 bp, Homo Sapiens
gcaagtacttacgcctccttggg

SEQ ID NO: 124 - DNA, 23 bp, Homo Sapiens
ttgcggtacatctccagcctggg

SEQ ID NO: 125 - DNA, 23 bp, Homo Sapiens
tttgcggtacatctccagcctgg

SEQ ID NO: 126 - DNA, 23 bp, Homo Sapiens
gcaaaacctgtccactcttatgg

SEQ ID NO: 127 - DNA, 23 bp, Homo Sapiens
ttggtgccataagagtggacagg

SEQ ID NO: 128 - DNA, 23 bp, Homo Sapiens
ggtgcaagtttcttatatgttgg

SEQ ID NO: 129 - DNA, 23 bp, Homo Sapiens
acctgatgcatataataatcagg

SEQ ID NO: 130 - DNA, 23 bp, Homo Sapiens
acctgattattatatgcatcagg

SEQ ID NO: 131 - DNA, 23 bp, Homo Sapiens
cagagcaccagagtgccgtctgg

SEQ ID NO: 132 - DNA, 23 bp, Homo Sapiens
agagcaccagagtgccgtctggg

SEQ ID NO: 133 - DNA, 23 bp, Homo Sapiens
agagtgccgtctgggtctgaagg

SEQ ID NO: 134 - DNA, 23 bp, Homo Sapiens
aggaaggccgtccattctcaggg

SEQ ID NO: 135 - DNA, 23 bp, Homo Sapiens
ggatagaaccaaccatgttgagg

SEQ ID NO: 136 - DNA, 23 bp, Homo Sapiens
tctgttgccctcaacatggttgg

SEQ ID NO: 137 - DNA, 23 bp, Homo Sapiens
ttagtctgttgccctcaacatgg

SEQ ID NO: 138 - DNA, 23 bp, Homo Sapiens
gtctggcaaatgggaggtgatgg

SEQ ID NO: 139 - DNA, 23 bp, Homo Sapiens
cagaggttctgtctggcaaatgg

SEQ ID NO: 140 - DNA, 23 bp, Homo Sapiens
ttgtagccagaggttctgtctgg

SEQ ID NO: 141 - DNA, 23 bp, Homo Sapiens
acttctggatgagctctctcagg

SEQ ID NO: 142 - DNA, 23 bp, Homo Sapiens
agagctcatccagaagtaaatgg

SEQ ID NO: 143 - DNA, 23 bp, Homo Sapiens
ttggtgtctccatttacttctgg

SEQ ID NO: 144 - DNA, 23 bp, Homo Sapiens
ttctggcttcccttcatacaggg

SEQ ID NO: 145 - DNA, 23 bp, Homo Sapiens
caggactcacacgactattctgg

SEQ ID NO: 146 - DNA, 23 bp, Homo Sapiens
ctactttcttgtgtaaagtcagg

SEQ ID NO: 147 - DNA, 23 bp, Homo Sapiens
gactttacacaagaaagtagagg

SEQ ID NO: 148 - DNA, 23 bp, Homo Sapiens
gtctttctccattagccttttgg

SEQ ID NO: 149 - DNA, 23 bp, Homo Sapiens
aatggagaaagacgtaacttcgg

SEQ ID NO: 150 - DNA, 23 bp, Homo Sapiens
atggagaaagacgtaacttcggg

SEQ ID NO: 151 - DNA, 23 bp, Homo Sapiens
tggagaaagacgtaacttcgggg

SEQ ID NO: 152 - DNA, 23 bp, Homo Sapiens
tttggttgactgctttcacctgg

SEQ ID NO: 153 - DNA, 23 bp, Homo Sapiens
tcactcaaatcggagacatttgg

SEQ ID NO: 154 - DNA, 23 bp, Homo Sapiens
atctgaagctctggattttcagg

SEQ ID NO: 155 - DNA, 23 bp, Homo Sapiens
gcttcagattctgaatgagcagg

SEQ ID NO: 156 - DNA, 23 bp, Homo Sapiens
cagattctgaatgagcaggaggg

SEQ ID NO: 157 - DNA, 23 bp, Homo Sapiens
aaggcagtgctaatgcctaatgg

SEQ ID NO: 158 - DNA, 23 bp, Homo Sapiens
gcagaaactgtagcaccattagg

SEQ ID NO: 159 - DNA, 23 bp, Homo Sapiens
accgcaatggaaacacaatctgg

SEQ ID NO: 160 - DNA, 23 bp, Homo Sapiens
tgtggttttctgcaccgcaatgg

SEQ ID NO: 161 - DNA, 23 bp, Homo Sapiens
cataaatgccattaacagtcagg

SEQ ID NO: 162 - DNA, 23 bp, Homo Sapiens
attagtagcctgactgttaatgg

SEQ ID NO: 163 - DNA, 23 bp, Homo Sapiens
cgatgggtgagtgatctcacagg

SEQ ID NO: 164 - DNA, 23 bp, Homo Sapiens
actcacccatcgcatacctcagg

SEQ ID NO: 165 - DNA, 23 bp, Homo Sapiens
ctcacccatcgcatacctcaggg

SEQ ID NO: 166 - DNA, 23 bp, Homo Sapiens
agcaacaggaggagttgcagagg

SEQ ID NO: 167 - DNA, 23 bp, Homo Sapiens
ccagtaggatcagcaacaggagg

SEQ ID NO: 168 - DNA, 23 bp, Homo Sapiens
ctcctgttgctgatcctactggg

SEQ ID NO: 169 - DNA, 23 bp, Homo Sapiens
ggcccagtaggatcagcaacagg

SEQ ID NO: 170 - DNA, 23 bp, Homo Sapiens
ttgctgatcctactgggccctgg

SEQ ID NO: 171 - DNA, 23 bp, Homo Sapiens
tggcaacagcttgcagctgtggg

SEQ ID NO: 172 - DNA, 23 bp, Homo Sapiens
cttgggtcccctgcttgcccggg

SEQ ID NO: 173 - DNA, 23 bp, Homo Sapiens
gtcccctgcttgcccgggaccgg

SEQ ID NO: 174 - DNA, 23 bp, Homo Sapiens
ctccggtcccgggcaagcagggg

SEQ ID NO: 175 - DNA, 23 bp, Homo Sapiens
tctccggtcccgggcaagcaggg

SEQ ID NO: 176 - DNA, 23 bp, Homo Sapiens
gtctccggtcccgggcaagcagg

SEQ ID NO: 177 - DNA, 23 bp, Homo Sapiens
gcttgcccgggaccggagacagg

SEQ ID NO: 178 - DNA, 23 bp, Homo Sapiens
ggtggcctgtctccggtcccggg

SEQ ID NO: 179 - DNA, 23 bp, Homo Sapiens
cggtggcctgtctccggtcccgg

SEQ ID NO: 180 - DNA, 23 bp, Homo Sapiens
catattcggtggcctgtctccgg

SEQ ID NO: 181 - DNA, 23 bp, Homo Sapiens
atctaggtactcatattcggtgg

SEQ ID NO: 182 - DNA, 23 bp, Homo Sapiens
ataatctaggtactcatattcgg

SEQ ID NO: 183 - DNA, 23 bp, Homo Sapiens
ttatgatttcctgccagaaacgg

SEQ ID NO: 184 - DNA, 23 bp, Homo Sapiens
atttctggaggctccgtttctgg

SEQ ID NO: 185 - DNA, 23 bp, Homo Sapiens
actgacaccactcctctgactgg

SEQ ID NO: 186 - DNA, 23 bp, Homo Sapiens
ctgacaccactcctctgactggg

SEQ ID NO: 187 - DNA, 23 bp, Homo Sapiens
accactcctctgactgggcctgg

SEQ ID NO: 188 - DNA, 23 bp, Homo Sapiens
aacccctgagtctaccactgtgg

SEQ ID NO: 189 - DNA, 23 bp, Homo Sapiens
ctccacagtggtagactcagggg

SEQ ID NO: 190 - DNA, 23 bp, Homo Sapiens
gctccacagtggtagactcaggg

SEQ ID NO: 191 - DNA, 23 bp, Homo Sapiens
ggctccacagtggtagactcagg

SEQ ID NO: 192 - DNA, 23 bp, Homo Sapiens
cctgctgcaaggcgttctactgg

SEQ ID NO: 193 - DNA, 23 bp, Homo Sapiens
ccagtagaacgccttgcagcagg

SEQ ID NO: 194 - DNA, 23 bp, Homo Sapiens
cgttctactggcctggatgcagg

SEQ ID NO: 195 - DNA, 23 bp, Homo Sapiens
tctactggcctggatgcaggagg

SEQ ID NO: 196 - DNA, 23 bp, Homo Sapiens
ccacggagctggccaacatgggg

SEQ ID NO: 197 - DNA, 23 bp, Homo Sapiens
cgtggacaggttccccatgttgg

SEQ ID NO: 198 - DNA, 23 bp, Homo Sapiens
gtccacggattcagcagctatgg

SEQ ID NO: 199 - DNA, 23 bp, Homo Sapiens
gaccactcaaccagtgcccacgg

SEQ ID NO: 200 - DNA, 23 bp, Homo Sapiens
ggagtggtctgtgcctccgtggg

SEQ ID NO: 201 - DNA, 23 bp, Homo Sapiens
ggcacagacaactcgactgacgg

SEQ ID NO: 202 - DNA, 23 bp, Homo Sapiens
gacaactcgactgacggccacgg

SEQ ID NO: 203 - DNA, 23 bp, Homo Sapiens
aactcgactgacggccacggagg

SEQ ID NO: 204 - DNA, 23 bp, Homo Sapiens
cacagaacccagtgccacagagg

SEQ ID NO: 205 - DNA, 23 bp, Homo Sapiens
ggtagtaggttccatggacaggg

SEQ ID NO: 206 - DNA, 23 bp, Homo Sapiens
tggtagtaggttccatggacagg

SEQ ID NO: 207 - DNA, 23 bp, Homo Sapiens
tcttttggtagtaggttccatgg

SEQ ID NO: 208 - DNA, 23 bp, Homo Sapiens
atggaacctactaccaaaagagg

SEQ ID NO: 209 - DNA, 23 bp, Homo Sapiens
aacagacctcttttggtagtagg

SEQ ID NO: 210 - DNA, 23 bp, Homo Sapiens
gggtatgaacagacctcttttgg

SEQ ID NO: 211 - DNA, 23 bp, Homo Sapiens
tgtgtcctctgttactcacaagg

SEQ ID NO: 212 - DNA, 23 bp, Homo Sapiens
gtgtcctctgttactcacaaggg

SEQ ID NO: 213 - DNA, 23 bp, Homo Sapiens
gtagttgacggacaaattgctgg

SEQ ID NO: 214 - DNA, 23 bp, Homo Sapiens
tttgtccgtcaactacccagtgg

SEQ ID NO: 215 - DNA, 23 bp, Homo Sapiens
ttgtccgtcaactacccagtggg

SEQ ID NO: 216 - DNA, 23 bp, Homo Sapiens
tgtccgtcaactacccagtgggg

SEQ ID NO: 217 - DNA, 23 bp, Homo Sapiens
gtccgtcaactacccagtggggg

SEQ ID NO: 218 - DNA, 23 bp, Homo Sapiens
ctctgtgaagcagtgcctgctgg

SEQ ID NO: 219 - DNA, 23 bp, Homo Sapiens
cctgctggccatcctaatcttgg

SEQ ID NO: 220 - DNA, 23 bp, Homo Sapiens
ccaagattaggatggccagcagg

SEQ ID NO: 221 - DNA, 23 bp, Homo Sapiens
ggccatcctaatcttggcgctgg

SEQ ID NO: 222 - DNA, 23 bp, Homo Sapiens
caccagcgccaagattaggatgg

SEQ ID NO: 223 - DNA, 23 bp, Homo Sapiens
agtgcacacgaagaagatagtgg

SEQ ID NO: 224 - DNA, 23 bp, Homo Sapiens
tatcttcttcgtgtgcactgtgg

SEQ ID NO: 225 - DNA, 23 bp, Homo Sapiens
cttcgtgtgcactgtggtgctgg

SEQ ID NO: 226 - DNA, 23 bp, Homo Sapiens
ggcggtccgcctctcccgcaagg

SEQ ID NO: 227 - DNA, 23 bp, Homo Sapiens
gcggtccgcctctcccgcaaggg

SEQ ID NO: 228 - DNA, 23 bp, Homo Sapiens
aattacgcacggggtacatgtgg

SEQ ID NO: 229 - DNA, 23 bp, Homo Sapiens
tgggggagtaattacgcacgggg

SEQ ID NO: 230 - DNA, 23 bp, Homo Sapiens
gtgggggagtaattacgcacggg

SEQ ID NO: 231 - DNA, 23 bp, Homo Sapiens
ggtgggggagtaattacgcacgg

SEQ ID NO: 232 - DNA, 23 bp, Homo Sapiens
taattactcccccaccgagatgg

SEQ ID NO: 233 - DNA, 23 bp, Homo Sapiens
agatgcagaccatctcggtgggg

SEQ ID NO: 234 - DNA, 23 bp, Homo Sapiens
gagatgcagaccatctcggtggg

SEQ ID NO: 235 - DNA, 23 bp, Homo Sapiens
tgagatgcagaccatctcggtgg

SEQ ID NO: 236 - DNA, 23 bp, Homo Sapiens
ggatgagatgcagaccatctcgg

SEQ ID NO: 237 - DNA, 23 bp, Homo Sapiens
atctcatccctgttgcctgatgg

SEQ ID NO: 238 - DNA, 23 bp, Homo Sapiens
tcatccctgttgcctgatggggg

SEQ ID NO: 239 - DNA, 23 bp, Homo Sapiens
ctcacccccatcaggcaacaggg

SEQ ID NO: 240 - DNA, 23 bp, Homo Sapiens
gagggcccctcacccccatcagg

SEQ ID NO: 241 - DNA, 23 bp, Homo Sapiens
gggccctctgccacagccaatgg

SEQ ID NO: 242 - DNA, 23 bp, Homo Sapiens
ccctctgccacagccaatggggg

SEQ ID NO: 243 - DNA, 23 bp, Homo Sapiens
cccccattggctgtggcagaggg

SEQ ID NO: 244 - DNA, 23 bp, Homo Sapiens
gcccccattggctgtggcagagg

SEQ ID NO: 245 - DNA, 23 bp, Homo Sapiens
ggacaggcccccattggctgtgg

SEQ ID NO: 246 - DNA, 23 bp, Homo Sapiens
ccgggctcttggccttggacagg

SEQ ID NO: 247 - DNA, 23 bp, Homo Sapiens
ctgtccaaggccaagagcccggg

SEQ ID NO: 248 - DNA, 23 bp, Homo Sapiens
tggcgtcaggcccgggctcttgg

SEQ ID NO: 249 - DNA, 23 bp, Homo Sapiens
cgggcctgacgccagagcccagg

SEQ ID NO: 250 - DNA, 23 bp, Homo Sapiens
caacaaccatgctgggcatctgg

SEQ ID NO: 251 - DNA, 23 bp, Homo Sapiens
gagggtccagatgcccagcatgg

SEQ ID NO: 252 - DNA, 23 bp, Homo Sapiens
catctggaccctcctacctctgg

SEQ ID NO: 253 - DNA, 23 bp, Homo Sapiens
agggctcaccagaggtaggaggg

SEQ ID NO: 254 - DNA, 23 bp, Homo Sapiens
ggagttgatgtcagtcacttggg

SEQ ID NO: 255 - DNA, 23 bp, Homo Sapiens
tggagttgatgtcagtcacttgg

SEQ ID NO: 256 - DNA, 23 bp, Homo Sapiens
agtgactgacatcaactccaagg

SEQ ID NO: 257 - DNA, 23 bp, Homo Sapiens
gtgactgacatcaactccaaggg

SEQ ID NO: 258 - DNA, 23 bp, Homo Sapiens
actccaagggattggaattgagg

SEQ ID NO: 259 - DNA, 23 bp, Homo Sapiens
cttcctcaattccaatcccttgg

SEQ ID NO: 260 - DNA, 23 bp, Homo Sapiens
tacagttgagactcagaacttgg

SEQ ID NO: 261 - DNA, 23 bp, Homo Sapiens
ttggaaggcctgcatcatgatgg

SEQ ID NO: 262 - DNA, 23 bp, Homo Sapiens
agaattggccatcatgatgcagg

SEQ ID NO: 263 - DNA, 23 bp, Homo Sapiens
gacagggcttatggcagaattgg

SEQ ID NO: 264 - DNA, 23 bp, Homo Sapiens
tgtaacatacctggaggacaggg

SEQ ID NO: 265 - DNA, 23 bp, Homo Sapiens
gtgtaacatacctggaggacagg

SEQ ID NO: 266 - DNA, 23 bp, Homo Sapiens
cgtacctgtgcaactcctgttgg

SEQ ID NO: 267 - DNA, 23 bp, Homo Sapiens
gatctactggaattcctaatggg

SEQ ID NO: 268 - DNA, 23 bp, Homo Sapiens
gagtcagctgttggcccattagg

SEQ ID NO: 269 - DNA, 23 bp, Homo Sapiens
ctgcctacaaactcagtctctgg

SEQ ID NO: 270 - DNA, 23 bp, Homo Sapiens
gggcaggcaggacggactccagg

SEQ ID NO: 271 - DNA, 23 bp, Homo Sapiens
ggagtccgtcctgcctgccctgg

SEQ ID NO: 272 - DNA, 23 bp, Homo Sapiens
gagtccgtcctgcctgccctggg

SEQ ID NO: 273 - DNA, 23 bp, Homo Sapiens
gaaaagggtccattggccaaagg

SEQ ID NO: 274 - DNA, 23 bp, Homo Sapiens
gcctgcagaaaagggtccattgg

SEQ ID NO: 275 - DNA, 23 bp, Homo Sapiens
ttgatgtgctacagggaacatgg

SEQ ID NO: 276 - DNA, 23 bp, Homo Sapiens
agcgttcttgatgtgctacaggg

SEQ ID NO: 277 - DNA, 23 bp, Homo Sapiens
cagcgttcttgatgtgctacagg

SEQ ID NO: 278 - DNA, 23 bp, Homo Sapiens
ctgtagcacatcaagaacgctgg

SEQ ID NO: 279 - DNA, 23 bp, Homo Sapiens
tgtagcacatcaagaacgctggg

SEQ ID NO: 280 - DNA, 23 bp, Homo Sapiens
ataggcaataatcatataacagg

SEQ ID NO: 281 - DNA, 23 bp, Homo Sapiens
agtgcgtttcgctgcaggtaagg

SEQ ID NO: 282 - DNA, 23 bp, Homo Sapiens
gagtgagtgcgtttcgctgcagg

SEQ ID NO: 283 - DNA, 23 bp, Homo Sapiens
gtcaggtttgtgcggttatgagg

SEQ ID NO: 284 - DNA, 23 bp, Homo Sapiens
cgctgctggtcaggtttgtgcgg

SEQ ID NO: 285 - DNA, 23 bp, Homo Sapiens
aaacctgaccagcagcgcagagg

SEQ ID NO: 286 - DNA, 23 bp, Homo Sapiens
ccagcagcgcagaggagccgtgg

SEQ ID NO: 287 - DNA, 23 bp, Homo Sapiens
ccacggctcctctgcgctgctgg

SEQ ID NO: 288 - DNA, 23 bp, Homo Sapiens
ccaactatctaactccactcagg

SEQ ID NO: 289 - DNA, 23 bp, Homo Sapiens
cctgagtggagttagatagttgg